European Patent Application EP 4 484 445 A1, published January 1, 2025. Title: HCMV NEUTRALIZING ANTIBODIES. Applicant: Universität zu Köln. Application EP. The sequence listing filed with the application follows.

SEQUENCE LISTING (120 sequences)

SEQ ID NO: 1 - protein, 8 aa, synthetic construct
  REGION 1..8: note = Heavy chain CS2it1p2_F7K CDR1
GYTLTDLS

SEQ ID NO: 2 - protein, 8 aa, synthetic construct
  REGION 1..8: note = Heavy chain CS2it1p2_F7K CDR2
FDPEHGEI

SEQ ID NO: 3 - protein, 21 aa, synthetic construct
  REGION 1..21: note = Heavy chain CS2it1p2_F7K CDR3
ATDSSIAMTGTYFSDLFALDV

SEQ ID NO: 4 - protein, 6 aa, synthetic construct
  REGION 1..6: note = Light chain CS2it1p2_F7K CDR1
QTINTN

SEQ ID NO: 5 - skipped

SEQ ID NO: 6 - protein, 9 aa, synthetic construct
  REGION 1..9: note = Light chain CS2it1p2_F7K CDR3
QQSHSPPHT

SEQ ID NO: 7 - protein, 8 aa, synthetic construct
  REGION 1..8: note = Heavy chain CS4tt1p1_E3K CDR1
GYTFDQYS

SEQ ID NO: 8 - protein, 8 aa, synthetic construct
  REGION 1..8: note = Heavy chain CS4tt1p1_E3K CDR2
ISSNGGSR

SEQ ID NO: 9 - protein, 18 aa, synthetic construct
  REGION 1..18: note = Heavy chain CS4tt1p1_E3K CDR3
ARAKKIFGGIIPPSGMDV

SEQ ID NO: 10 - protein, 6 aa, synthetic construct
  REGION 1..6: note = Light chain CS4tt1p1_E3K CDR1
QNIYNW

SEQ ID NO: 11 - skipped

SEQ ID NO: 12 - protein, 10 aa, synthetic construct
  REGION 1..10: note = Light chain CS4tt1p1_E3K CDR3
QHYYNYPPWT

SEQ ID NO: 13 - protein, 8 aa, synthetic construct
  REGION 1..8: note = Heavy chain CS1pt2p3_E1K CDR1
GYSFNTYP

SEQ ID NO: 14 - protein, 8 aa, synthetic construct
  REGION 1..8: note = Heavy chain CS1pt2p3_E1K CDR2
INTYKGDT

SEQ ID NO: 15 - protein, 11 aa, synthetic construct
  REGION 1..11: note = Heavy chain CS1pt2p3_E1K CDR3
AKEDPWGWLEY

SEQ ID NO: 16 - protein, 6 aa, synthetic construct
  REGION 1..6: note = Light chain CS1pt2p3_E1K CDR1
QGISSY

SEQ ID NO: 17 - skipped

SEQ ID NO: 18 - protein, 9 aa, synthetic construct
  REGION 1..9: note = Light chain CS1pt2p3_E1K CDR3
QQYSTYAYT

SEQ ID NO: 19 - protein, 8 aa, synthetic construct
  REGION 1..8: note = Heavy chain CS2pt1p2_E12K CDR1
GESLTDKC

SEQ ID NO: 20 - protein, 7 aa, synthetic construct
  REGION 1..7: note = Heavy chain CS2pt1p2_E12K CDR2
IDHMDTT

SEQ ID NO: 21 - protein, 22 aa, synthetic construct
  REGION 1..22: note = Heavy chain CS2pt1p2_E12K CDR3
ARGGPSLKTVYGVVFLHNFFDT

SEQ ID NO: 22 - protein, 12 aa, synthetic construct
  REGION 1..12: note = Light chain CS2pt1p2_E12K CDR1
QSLLYRSENKNY

SEQ ID NO: 23 - skipped

SEQ ID NO: 24 - protein, 9 aa, synthetic construct
  REGION 1..9: note = Light chain CS2pt1p2_E12K CDR3
QQYYRAPWT

SEQ ID NO: 25 - protein, 8 aa, synthetic construct
  REGION 1..8: note = Heavy chain CS2pt1p2_A10L CDR1
GFSFSDYY

SEQ ID NO: 26 - protein, 8 aa, synthetic construct
  REGION 1..8: note = Heavy chain CS2pt1p2_A10L CDR2
ISPSGSPT

SEQ ID NO: 27 - protein, 16 aa, synthetic construct
  REGION 1..16: note = Heavy chain CS2pt1p2_A10L CDR3
ARDNTVFGVVTTPMDH

SEQ ID NO: 28 - protein, 8 aa, synthetic construct
  REGION 1..8: note = Light chain CS2pt1p2_A10L CDR1
SSNIGSNT

SEQ ID NO: 29 - skipped

SEQ ID NO: 30 - protein, 11 aa, synthetic construct
  REGION 1..11: note = Light chain CS2pt1p2_A10L CDR3
AAWDDSLNGRV

SEQ ID NO: 31 - protein, 10 aa, synthetic construct
  REGION 1..10: note = Heavy chain CS2tt1p1_C11L CDR1
AGSVRSDRYY

SEQ ID NO: 32 - protein, 7 aa, synthetic construct
  REGION 1..7: note = Heavy chain CS2tt1p1_C11L CDR2
LYFGGTN

SEQ ID NO: 33 - protein, 11 aa, synthetic construct
  REGION 1..11: note = Heavy chain CS2tt1p1_C11L CDR3
AAALTTVTFIS

SEQ ID NO: 34 - protein, 9 aa, synthetic construct
  REGION 1..9: note = Light chain CS2tt1p1_C11L CDR1
SGINVGTYR

SEQ ID NO: 35 - protein, 7 aa, synthetic construct
  REGION 1..7: note = Light chain CS2tt1p1_C11L CDR2
YKSDSDK

SEQ ID NO: 36 - protein, 9 aa, synthetic construct
  REGION 1..9: note = Light chain CS2tt1p1_C11L CDR3
MIWHNSVVV

SEQ ID NO: 37 - protein, 8 aa, synthetic construct
  REGION 1..8: note = Heavy chain CS3tt1p3_A12K CDR1
GFTFTDYY

SEQ ID NO: 38 - protein, 8 aa, synthetic construct
  REGION 1..8: note = Heavy chain CS3tt1p3_A12K CDR2
ISSSGSYT

SEQ ID NO: 39 - protein, 10 aa, synthetic construct
  REGION 1..10: note = Heavy chain CS3tt1p3_A12K CDR3
ARSPMKRLDF

SEQ ID NO: 40 - protein, 6 aa, synthetic construct
  REGION 1..6: note = Light chain CS3tt1p3_A12K CDR1
QSVGST

SEQ ID NO: 41 - skipped

SEQ ID NO: 42 - protein, 10 aa, synthetic construct
  REGION 1..10: note = Light chain CS3tt1p3_A12K CDR3
QHYESWPPWT

SEQ ID NO: 43 - protein, 8 aa, synthetic construct
  REGION 1..8: note = Heavy chain CS3pt1p1_E4K CDR1
GYTFSNYG

SEQ ID NO: 44 - protein, 8 aa, synthetic construct
  REGION 1..8: note = Heavy chain CS3pt1p1_E4K CDR2
ISGYNGNT

SEQ ID NO: 45 - protein, 15 aa, synthetic construct
  REGION 1..15: note = Heavy chain CS3pt1p1_E4K CDR3
AREGSRPYYYRGMDV

SEQ ID NO: 46 - protein, 6 aa, synthetic construct
  REGION 1..6: note = Light chain CS3pt1p1_E4K CDR1
QSISSY

SEQ ID NO: 47 - skipped

SEQ ID NO: 48 - protein, 10 aa, synthetic construct
  REGION 1..10: note = Light chain CS3pt1p1_E4K CDR3
QQRGMSLPWT

SEQ ID NO: 49 - protein, 8 aa, synthetic construct
  REGION 1..8: note = Heavy chain CS2tt1p3_C3K CDR1
GGSISNYY

SEQ ID NO: 50 - protein, 7 aa, synthetic construct
  REGION 1..7: note = Heavy chain CS2tt1p3_C3K CDR2
IYYSGST

SEQ ID NO: 51 - protein, 20 aa, synthetic construct
  REGION 1..20: note = Heavy chain CS2tt1p3_C3K CDR3
ARQRTPNYYGSGSFSNWFDP

SEQ ID NO: 52 - protein, 12 aa, synthetic construct
  REGION 1..12: note = Light chain CS2tt1p3_C3K CDR1
QSVLFSSNNKNY

SEQ ID NO: 53 - skipped

SEQ ID NO: 54 - protein, 9 aa, synthetic construct
  REGION 1..9: note = Light chain CS2tt1p3_C3K CDR3
QQYYGLPST

SEQ ID NO: 55 - protein, 10 aa, synthetic construct
  REGION 1..10: note = Heavy chain CS2pt1p3_E12K CDR1
GDSVSNNDAA

SEQ ID NO: 56 - protein, 9 aa, synthetic construct
  REGION 1..9: note = Heavy chain CS2pt1p3_E12K CDR2
THYRSRWYN

SEQ ID NO: 57 - protein, 24 aa, synthetic construct
  REGION 1..24: note = Heavy chain CS2pt1p3_E12K CDR3
ARGTPSPKDYSDGGGYYYVEYFQD

SEQ ID NO: 58 - protein, 6 aa, synthetic construct
  REGION 1..6: note = Light chain CS2pt1p3_E12K CDR1
QSVSTD

SEQ ID NO: 59 - skipped

SEQ ID NO: 60 - protein, 11 aa, synthetic construct
  REGION 1..11: note = Light chain CS2pt1p3_E12K CDR3
QQRTNWPLAYT

SEQ ID NO: 61 - protein, 8 aa, synthetic construct
  REGION 1..8: note = Heavy chain CS3tt1p1_G9K CDR1
GYTFSNYW

SEQ ID NO: 62 - protein, 8 aa, synthetic construct
  REGION 1..8: note = Heavy chain CS3tt1p1_G9K CDR2
IYPGDSDT

SEQ ID NO: 63 - protein, 19 aa, synthetic construct
  REGION 1..19: note = Heavy chain CS3tt1p1_G9K CDR3
GLGLAAGGRFYYYYHGMDV

SEQ ID NO: 64 - protein, 12 aa, synthetic construct
  REGION 1..12: note = Light chain CS3tt1p1_G9K CDR1
QSVFYSSNNKDY

SEQ ID NO: 65 - skipped

SEQ ID NO: 66 - protein, 8 aa, synthetic construct
  REGION 1..8: note = Light chain CS3tt1p1_G9K CDR3
QQYYTTPQ

SEQ ID NO: 67 - protein, 8 aa, synthetic construct
  REGION 1..8: note = Heavy chain CS3tt1p4_G2K CDR1
GFTFSDYY

SEQ ID NO: 68 - protein, 8 aa, synthetic construct
  REGION 1..8: note = Heavy chain CS3tt1p4_G2K CDR2
ISSASSYI

SEQ ID NO: 69 - protein, 10 aa, synthetic construct
  REGION 1..10: note = Heavy chain CS3tt1p4_G2K CDR3
ARSPMKVLDH

SEQ ID NO: 70 - protein, 6 aa, synthetic construct
  REGION 1..6: note = Light chain CS3tt1p4_G2K CDR1
QSVDNR

SEQ ID NO: 71 - skipped

SEQ ID NO: 72 - protein, 10 aa, synthetic construct [sequence omitted]

SEQ ID NO: 73 - protein, 8 aa, synthetic construct
  REGION 1..8: note = Heavy chain CS3tt1p1_A9K CDR1
GFSFSAYA

SEQ ID NO: 74 - protein, 8 aa, synthetic construct
  REGION 1..8: note = Heavy chain CS3tt1p1_A9K CDR2
IWFDGSKK

SEQ ID NO: 75 - protein, 10 aa, synthetic construct
  REGION 1..10: note = Heavy chain CS3tt1p1_A9K CDR3
SREEYRSFNY

SEQ ID NO: 76 - protein, 6 aa, synthetic construct
  REGION 1..6: note = Light chain CS3tt1p1_A9K CDR1
RSIGTN

SEQ ID NO: 77 - skipped

SEQ ID NO: 78 - protein, 9 aa, synthetic construct
  REGION 1..9: note = Light chain CS3tt1p1_A9K CDR3
QQSYSTPRT

SEQ ID NO: 79 - protein, 8 aa, synthetic construct
  REGION 1..8: note = Heavy chain CS2pt1p1_E1K CDR1
GRSMNDFY

SEQ ID NO: 80 - protein, 7 aa, synthetic construct
  REGION 1..7: note = Heavy chain CS2pt1p1_E1K CDR2
IYYTGST

SEQ ID NO: 81 - protein, 20 aa, synthetic construct
  REGION 1..20: note = Heavy chain CS2pt1p1_E1K CDR3
ARQRTPNYFASGTYSNWFDP

SEQ ID NO: 82 - protein, 12 aa, synthetic construct
  REGION 1..12: note = Light chain CS2pt1p1_E1K CDR1
QSLLYSANNKNY

SEQ ID NO: 83 - skipped

SEQ ID NO: 84 - protein, 9 aa, synthetic construct
  REGION 1..9: note = Light chain CS2pt1p1_E1K CDR3
QQYFATPPT

SEQ ID NO: 85 - protein, 128 aa, synthetic construct
  REGION 1..128: note = Heavy chain variable domain CS2it1p2_F7K [organism=Artificial Sequence]
QVQLVQSGAEVKKPGASVRVSCKVSGYTLTDLSIHWVRQAPGKGLEWMGGFDPEHGEIMYAQKFQGRVTVTEDTSTHTTYMEVNSLRSEDTAVYYCATDSSIAMTGTYFSDLFALDVWGQGTTVIVSS

SEQ ID NO: 86 - protein, 107 aa, synthetic construct
  REGION 1..107: note = Light chain variable domain CS2it1p2_F7K [organism=Artificial Sequence]
DIQMTQSPSSLSASVGDRVTITCRASQTINTNLNWYQQKPGKAPRLLIFGTFSLKSGVPSRFSGGGSGTDFTLTISSLQPEDFAAYFCQQSHSPPHTFGQGTKLELK

SEQ ID NO: 87 - protein, 125 aa, synthetic construct
  REGION 1..125: note = Heavy chain variable domain CS4tt1p1_E3K [organism=Artificial Sequence]
EVRLVESGGGFVQTGGSLRLSCAASGYTFDQYSMHWVRQVPGKGLQFVSTISSNGGSRYYADSVKGRFVVSRDEEKEVLYLQMGRLRTDDTGIYFCARAKKIFGGIIPPSGMDVWGRGTTVTVSS

SEQ ID NO: 88 - protein, 105 aa, synthetic construct
  REGION 1..105: note = Light chain variable domain CS4tt1p1_E3K [organism=Artificial Sequence]
DIQLTQSPSSLSASVGDRVTITCRASQNIYNWLAWYQQKPGQAPKLLIFDASTLEGGVPSRFGGSGSGTDFTLTISNLRPEDFATYFCQHYYNYPPWTFGQGTKV

SEQ ID NO: 89 - protein, 118 aa, synthetic construct
  REGION 1..118: note = Heavy chain variable domain CS1pt2p3_E1K [organism=Artificial Sequence]
QVQLVQSGVEVKKPGAAVKVSCKASGYSFNTYPIAWVRQAPGEGLEWIGRINTYKGDTKYLQRLQGRVAMTIDISTATAYMELRSLRSDDTAVYFCAKEDPWGWLEYWGQGTPVTVSS

SEQ ID NO: 90 - protein, 107 aa, synthetic construct
  REGION 1..107: note = Light chain variable domain CS1pt2p3_E1K [organism=Artificial Sequence]
DIQMTQSPSTLSASVGDRVTITCRASQGISSYLAWYQQKPGKAPNLLIFGASTLQSGVPSRFSGSGSGTDFTLTISSLQPDDFATYYCQQYSTYAYTFGQGTRLEIK

SEQ ID NO: 91 - protein, 128 aa, synthetic construct
  REGION 1..128: note = Heavy chain variable domain CS2pt1p2_E12K [organism=Artificial Sequence]
QVQLQQWGAGLLRPSETLSLTCAVYGESLTDKCWTWIRQAPGKGLEWIGDIDHMDTTKYNPSLKSRVTISVDGSKNQFSLRLDSVTAADTGVYYCARGGPSLKTVYGVVFLHNFFDTWGQGTRVVVSS

SEQ ID NO: 92 - protein, 113 aa, synthetic construct
  REGION 1..113: note = Light chain variable domain CS2pt1p2_E12K [organism=Artificial Sequence]
DVVMTQSPDSLALSLGERATINCKSSQSLLYRSENKNYLAWYQQKPGQSPRLLISWASDRHSGVPERFSGSGSDTDFILTINSLQAEDVAVYYCQQYYRAPWTFGQGTKVEVK

SEQ ID NO: 93 - protein, 123 aa, synthetic construct
  REGION 1..123: note = Heavy chain variable domain CS2pt1p2_A10L [organism=Artificial Sequence]
QVHLEESGGGLVKPGGSLRLSCVASGFSFSDYYMSWIRQAPGKGLEWLSYISPSGSPTSNADSMKGRFTISRDNARSSLYLQVHSLRVEDTAVYYCARDNTVFGVVTTPMDHWGQGTLVTVSS

SEQ ID NO: 94 - protein, 109 aa, synthetic construct
  REGION 1..109: note = Light chain variable domain CS2pt1p2_A10L [organism=Artificial Sequence]
QSALTQPPSASGTPGQRVTISCSGSSSNIGSNTVHWYQQLPGTAPKLLIYSNNQRPSGVPDRFSGSRSGTSASLAISGLRSEDEADYYCAAWDDSLNGRVFGTGTKVTV

SEQ ID NO: 95 - protein, 118 aa, synthetic construct
  REGION 1..118: note = Heavy chain variable domain CS2tt1p1_C11L [organism=Artificial Sequence]
QVQLQESGPGLMRPSETLSLTCTVSAGSVRSDRYYWTWIRQHPGKGLEWIGYLYFGGTNYYNPSLKSRVTISVDASKNQFSLRLTSVTAADTARYYCAAALTTVTFISWGQGAQVTVA

SEQ ID NO: 96 - protein, 115 aa, synthetic construct
  REGION 1..115: note = Light chain variable domain CS2tt1p1_C11L [organism=Artificial Sequence]
QAVLTQPSSLSASPGASASLTCTLHSGINVGTYRIYWYQQKPGSPPQYLLRYKSDSDKQRGSGVPSRFSGSKDASANAGRLVISGLQSEDEADYFCMIWHNSVVVFGGGTKLTVL

SEQ ID NO: 97 - protein, 117 aa, synthetic construct
  REGION 1..117: note = Heavy chain variable domain CS3tt1p3_A12K [organism=Artificial Sequence]
QVQLVQSGGGLVKPGGSLRLSCAASGFTFTDYYMSWIRQSPGKGLEWISYISSSGSYTFYPDSVKGRFTVSRDNTKNSLFLQMDRLRVEDTAVYYCARSPMKRLDFWGQGVLVTVSS

SEQ ID NO: 98 - protein, 107 aa, synthetic construct
  REGION 1..107: note = Light chain variable domain CS3tt1p3_A12K [organism=Artificial Sequence]
EIVMTQSPATLSLSPGERATLSCRASQSVGSTLAWYQQKPGQAPRLLIFGTSTRATGVPTRFSGSGSGTEFTLIISSLRSEDSGLYFCQHYESWPPWTFGQGTKVEV

SEQ ID NO: 99 - protein, 122 aa, synthetic construct
  REGION 1..122: note = Heavy chain variable domain CS3pt1p1_E4K [organism=Artificial Sequence]
QVHLVQSGAEVKKPGASVKVSCKASGYTFSNYGISWVRQAPGQGLEWMGWISGYNGNTNYAQKFKDRVIMSTDPFTSTVYLEVRSLRSDDTAVYYCAREGSRPYYYRGMDVWGQGTTVTVSS

SEQ ID NO: 100 - protein, 108 aa, synthetic construct
  REGION 1..108: note = Light chain variable domain CS3pt1p1_E4K [organism=Artificial Sequence]
EIVLTQFPATLSLSPGERATLFCRASQSISSYVAWYQHKPGQAPRLLIYDTVSRATGVPARFSGAGSGTDFTLSISSLESGDFGVYYCQQRGMSLPWTFGQGTKVEIK

SEQ ID NO: 101 - protein, 126 aa, synthetic construct
  REGION 1..126: note = Heavy chain variable domain CS2tt1p3_C3K [organism=Artificial Sequence]
QVQLQESGPGLVKPSETLSLTCTVSGGSISNYYWNWIRQPPGKRLEWIGYIYYSGSTNYNPSLKSRVSIAVDTSKKQFSLKLSSVTAADTAVYYCARQRTPNYYGSGSFSNWFDPWGQGTLVTVSS

SEQ ID NO: 102 - protein, 113 aa, synthetic construct
  REGION 1..113: note = Light chain variable domain CS2tt1p3_C3K [organism=Artificial Sequence]
DIVMTQSPDSLAVSLGERATINCKSSQSVLFSSNNKNYLSWYQQKPGQPPKLLIYWASTRESGVPDRFSGSGSGTDFTLTITRLQAEDVAVYYCQQYYGLPSTFGQGTKVEIK

SEQ ID NO: 103 - protein, 134 aa, synthetic construct
  REGION 1..134: note = Heavy chain variable domain CS2pt1p3_E12K [organism=Artificial Sequence]
QVQLQQSGPGLVKPSQTLSLTCVISGDSVSNNDAAWFWIRQSPSRGLEWLGRTHYRSRWYNDYAVSVKSRIRINPDTSKNLFSLHLNSMTPEDSAVYFCARGTPSPKDYSDGGGYYYVEYFQDWGQGTLVTVSS

SEQ ID NO: 104 - protein, 109 aa, synthetic construct
  REGION 1..109: note = Light chain variable domain CS2pt1p3_E12K [organism=Artificial Sequence]
EIVLTQSPATLSVSPGERATLSCRASQSVSTDLAWYQQKPGQAPRLLIHDASTRATGIPARFTGSGSGTDFTLTISSLEPEDFAVYYCQQRTNWPLAYTFGRGTKLEIK

SEQ ID NO: 105 - protein, 126 aa, synthetic construct
  REGION 1..126: note = Heavy chain variable domain CS3tt1p1_G9K [organism=Artificial Sequence]
EVQLVQSGTEVKKPGESLRISCKGSGYTFSNYWIAWVRQRPGKGLEWMGLIYPGDSDTRYSPSIQGQVSLSADKSISTAYLQWTSLKASDTAVYYCGLGLAAGGRFYYYYHGMDVWGQGTTVIVSS

SEQ ID NO: 106 - protein, 112 aa, synthetic construct
  REGION 1..112: note = Light chain variable domain CS3tt1p1_G9K [organism=Artificial Sequence]
DIVLTQSPDSLAVSLGETATINCRSSQSVFYSSNNKDYLAWYQHKPGQPPKLLIYWASTRESGVPDRFSGSGSGTDFTLTISSLQAEDVAIYYCQQYYTTPQFGQGTKVEIK

SEQ ID NO: 107 - protein, 117 aa, synthetic construct
  REGION 1..117: note = Heavy chain variable domain CS3tt1p4_G2K [organism=Artificial Sequence]
QVHLVESGGGLVKPGGSLRLSCAASGFTFSDYYMSWIRQTPGKGLEWIAYISSASSYIHYADSVKGRFTVSRDNVHNTLSLLMNGLRVEDTAMYYCARSPMKVLDHWGQGTVVTVSS

SEQ ID NO: 108 - protein, 107 aa, synthetic construct
  REGION 1..107: note = Light chain variable domain CS3tt1p4_G2K [organism=Artificial Sequence]
EIVMTQSPATLSVSPGERVTLSCRASQSVDNRLAWYQQKPGQPPRLLISGASTRATGIPARFSGSGSGTEFTLTISGLQSEDSAIYYCQQYNNWPPWTFGQGTKVEI

SEQ ID NO: 109 - protein, 116 aa, synthetic construct
  REGION 1..116: note = Heavy chain variable domain CS3tt1p1_A9K [organism=Artificial Sequence]
QVQLVESGGGVVQPGRSLRLSCAASGFSFSAYAMHWVRQAPGRGLEWVAVIWFDGSKKVYADSVKGRFTISRDNSKNTLHLQMDSLRAEDTAVYYCSREEYRSFNYWGQGTLVTVS

SEQ ID NO: 110 - protein, 107 aa, synthetic construct
  REGION 1..107: note = Light chain variable domain CS3tt1p1_A9K [organism=Artificial Sequence]
DIQMTQSPSSLSASVGDRVTIICRASRSIGTNLNWYQQRVGKAPNLLIYDASRLHSGVPSRFSGSGTGTAFTLTISSLQPEDFATYYCQQSYSTPRTFGPGTKVDSK

SEQ ID NO: 111 - protein, 125 aa, synthetic construct
  REGION 1..125: note = Heavy chain variable domain CS2pt1p1_E1K [organism=Artificial Sequence]
QVRLQESGPGLIKPSETLSLTCTVSGRSMNDFYWNWIRQPPGKGLEWIGHIYYTGSTTYNPSLESRVVISLDTSKNLFSLQLRSVTAADTALYYCARQRTPNYFASGTYSNWFDPWGQGIGVTVS

SEQ ID NO: 112 - protein, 113 aa, synthetic construct
  REGION 1..113: note = Light chain variable domain CS2pt1p1_E1K [organism=Artificial Sequence]
DIVMTQSPDSLAVSLGERATINCKSSQSLLYSANNKNYLAWYQQKPGQPPKLLIYWASTRESGVPDRFSGSGSGTDFTLTINSLQAADVAVYSCQQYFATPPTSGQGTKVALK

SEQ ID NO: 113 - protein, 8 aa, synthetic construct
  REGION 1..8: note = Heavy chain CS3pt1p4_C1L CDR1
GGTFTDYA

SEQ ID NO: 114 - protein, 8 aa, synthetic construct
  REGION 1..8: note = Heavy chain CS3pt1p4_C1L CDR2
IIPVLGTP

SEQ ID NO: 115 - protein, 15 aa, synthetic construct
  REGION 1..15: note = Heavy chain CS3pt1p4_C1L CDR3
ARGVTHPYYYYAMDV

SEQ ID NO: 116 - protein, 9 aa, synthetic construct
  REGION 1..9: note = Light chain CS3pt1p4_C1L CDR1
SSDVGAYDY

SEQ ID NO: 117 - skipped

SEQ ID NO: 118 - protein, 12 aa, synthetic construct
  REGION 1..12: note = Light chain CS3pt1p4_C1L CDR3
GSYTSSSAFFYV

SEQ ID NO: 119 - protein, 122 aa, synthetic construct
  REGION 1..122: note = Heavy chain variable domain CS3pt1p4_C1L [organism=Artificial Sequence]
QVQLVQSGAEVKKPGSSVKVSCKASGGTFTDYALSWVRQAPGQGLEWMGGIIPVLGTPHYAQKFEDRVTIIADESTGTVFMALSSLRSDDTGMYYCARGVTHPYYYYAMDVWGQGTTITVSS

SEQ ID NO: 120 - protein, 112 aa, synthetic construct
  REGION 1..112: note = Light chain variable domain CS3pt1p4_C1L [organism=Artificial Sequence]
QSALTQPASVSGSPGQSISISCTGTSSDVGAYDYVSWYQQHPGKAPRLIIYDVNKRPSGVPYRFSGSKSGTAASLTISGLQSEDEAVYYCGSYTSSSAFFYVFGTGMVTVLG